European Patent Application EP 4 786 490 A1, published August 5, 2026. Title: 糖苷内切酶S2突变体、其制备方法及其在抗体糖基化改造中的应用. Applicant: 上海糖岭生物医药有限责任公司. The sequence listing filed with the application follows.

SEQUENCE LISTING (10 sequences)

SEQ ID NO: 1 - protein, 843 aa, synthetic construct
MDKHLLVKRTLGCVCAATLMGAALATHHDSLNTVKAEEKTVQTGKTDQQVGAKLVQEIREGKRGPLYAGYFRTWHDRASTGIDGKQQHPENTMAEVPKEVDILFVFHDHTASDSPFWSELKDSYVHKLHQQGTALVQTIGVNELNGRTGLSKDYPDTPEGNKALAAAIVKAFVTDRGVDGLDIDIEHEFTNKRTPEEDARALNVFKEIAQLIGKNGSDKSKLLIMDTTLSVENNPIFKGIAEDLDYLLRQYYGSQGGEAEVDTINSDWNQYQNYIDASQFMIGFSFFEESASKGNLWFDVNEYDPNNPEKGKDIEGTRAKKYAEWQPSTGGLKAGIFSYAIDRDGVAHVPSTYKNRTSTNLQRHEVDNISHTDYTVSRKLKTLMTEDKRYDVIDQKDIPDPALREQIIQQVGQYKGDLERYNKTLVLTGDKIQNLKGLEKLSKLQKLELRQLSNVKEITPELLPESMKKDAELVMVGMTGLEKLNLSGLNRQTLDGIDVNSITHLTSFDISHNSLDLSEKSEDRKLLMTLMEQVSNHQKITVKNTAFENQKPKGYYPQTYDTKEGHYDVDNAEHDILTDFVFGTVTKRNTFIGDEEAFAIYKEGAVDGRQYVSKDYTYEAFRKDYKGYKVHLTASNLGETVTSKVTATTDETYLVDVSDGEKVVHHMKLNIGSGAIMMENLAKGAKVIGTSGDFEQAKKIFDGEKSDRFFTWGQTNWIAFDLGEINLAKEWRLFNAETNTEIKTDSSLNVAKGRLQILKDTTIDLEKMDIKNRKEYLSNDENWTDVAQMDDAKAIFNSKLSNVLSRYWRFCVDGGASSYYPQYTELQILGQRLSNDVANTLKD

SEQ ID NO: 2 - protein, 995 aa, synthetic construct
MDKHLLVKRTLGCVCAATLMGAALATHHDSLNTVKAEEKTVQVQKGLPSIDSLHYLSENSKKEFKEELSKAGQESQKVKEILAKAQQADKQAQELAKMKIPEKIPMKPLHGPLYGGYFRTWHDKTSDPTEKDKVNSMGELPKEVDLAFIFHDWTKDYSLFWKELATKHVPKLNKQGTRVIRTIPWRFLAGGDNSGIAEDTSKYPNTPEGNKALAKAIVDEYVYKYNLDGLDVDVEHDSIPKVDKKEDTAGVERSIQVFEEIGKLIGPKGVDKSRLFIMDSTYMADKNPLIERGAPYINLLLVQVYGSQGEKGGWEPVSNRPEKTMEERWQGYSKYIRPEQYMIGFSFYEENAQEGNLWYDINSRKDEDKANGINTDITGTRAERYARWQPKTGGVKGGIFSYAIDRDGVAHQPKKYAKQKEFKDATDNIFHSDYSVSKALKTVMLKDKSYDLIDEKDFPDKALREAVMAQVGTRKGDLERFNGTLRLDNPAIQSLEGLNKFKKLAQLDLIGLSRITKLDRSVLPANMKPGKDTLETVLETYKKDNKEEPATIPPVSLKVSGLTGLKELDLSGFDRETLAGLDAATLTSLEKVDISGNKLDLAPGTENRQIFDTMLSTISNHVGSNEQTVKFDKQKPTGHYPDTYGKTSLRLPVANEKVDLQSQLLFGTVTNQGTLINSEADYKAYQNHKIAGRSFVDSNYHYNNFKVSYENYTVKVTDSTLGTTTDKTLATDKEETYKVDFFSPADKTKAVHTAKVIVGDEKTMMVNLAEGATVIGGSADPVNARKVFDGQLGSETDNISLGWDSKQSIIFKLKEDGLIKHWRFFNDSARNPETTNKPIQEASLQIFNIKDYNLDNLLENPNKFDDEKYWITVDTYSAQGERATAFSNTLNNITSKYWRVVFDTKGDRYSSPVVPELQILGYPLPNADTIMKTVTTAKELSQQKDKFSQKMLDELKIKEMALETSLNSKIFDVTAINANAGVLKDCIEKRQLLKK

SEQ ID NO: 3 - protein, 894 aa, synthetic construct
EEKTVQVQKGLPSIDSLHYLSENSKKEFKEELSKAGQESQKVKEILAKAQQADKQAQELAKMKIPEKIPMKPLHGPLYGGYFRTWHDKTSDPTEKDKVNSMGELPKEVDLAFIFHDWTKDYSLFWKELATKHVPKLNKQGTRVIRTIPWRFLAGGDNSGIAEDTSKYPNTPEGNKALAKAIVDEYVYKYNLDGLDVDVEHDSIPKVDKKEDTAGVERSIQVFEEIGKLIGPKGVDKSRLFIMDSTYMADKNPLIERGAPYINLLLVQVYGSQGEKGGWEPVSNRPEKTMEERWQGYSKYIRPEQYMIGFSFYEENAQEGNLWYDINSRKDEDKANGINTDITGTRAERYARWQPKTGGVKGGIFSYAIDRDGVAHQPKKYAKQKEFKDATDNIFHSDYSVSKALKTVMLKDKSYDLIDEKDFPDKALREAVMAQVGTRKGDLERFNGTLRLDNPAIQSLEGLNKFKKLAQLDLIGLSRITKLDRSVLPANMKPGKDTLETVLETYKKDNKEEPATIPPVSLKVSGLTGLKELDLSGFDRETLAGLDAATLTSLEKVDISGNKLDLAPGTENRQIFDTMLSTISNHVGSNEQTVKFDKQKPTGHYPDTYGKTSLRLPVANEKVDLQSQLLFGTVTNQGTLINSEADYKAYQNHKIAGRSFVDSNYHYNNFKVSYENYTVKVTDSTLGTTTDKTLATDKEETYKVDFFSPADKTKAVHTAKVIVGDEKTMMENLAKGAKVIGTSGDFEQAKKIFDGEKSDRFFTWGQTNWIAFDLGEINLAKEWRLFNAETNTEIKTDSSLNVAKGRLQILKDTTIDLEKMDIKNRKEYLSNDENWTDVAQMDDAKAIFNSKLSNVLSRYWRFCVDGGASSYYPQYTELQILGQRLSNDVANTLKD

SEQ ID NO: 4 - protein, 810 aa, synthetic construct
EEKTVQTGKTDQQVGAKLVQEIREGKRGPLYAGYFRTWHDRASTGIDGKQQHPENTMAEVPKEVDILFVFHDHTASDSPFWSELKDSYVHKLHQQGTALVQTIGVNELNGRTGLSKDYPDTPEGNKALAAAIVKAFVTDRGVDGLDIDIEHEFTNKRTPEEDARALNVFKEIAQLIGKNGSDKSKLLIMDTTLSVENNPIFKGIAEDLDYLLRQYYGSQGGEAEVDTINSDWNQYQNYIDASQFMIGFSFFEESASKGNLWFDVNEYDPNNPEKGKDIEGTRAKKYAEWQPSTGGLKAGIFSYAIDRDGVAHVPSTYKNRTSTNLQRHEVDNISHTDYTVSRKLKTLMTEDKRYDVIDQKDIPDPALREQIIQQVGQYKGDLERYNKTLVLTGDKIQNLKGLEKLSKLQKLELRQLSNVKEITPELLPESMKKDAELVMVGMTGLEKLNLSGLNRQTLDGIDVNSITHLTSFDISHNSLDLSEKSEDRKLLMTLMEQVSNHQKITVKNTAFDKQKPTGHYPDTYGKTSLRLPVANEKVDLQSQLLFGTVTNQGTLINSEADYKAYQNHKIAGRSFVDSNYHYNNFKVSYENYTVKVTDSTLGTTTDKTLATDKEETYKVDFFSPADKTKAVHTAKVIVGDEKTMMENLAKGAKVIGTSGDFEQAKKIFDGEKSDRFFTWGQTNWIAFDLGEINLAKEWRLFNAETNTEIKTDSSLNVAKGRLQILKDTTIDLEKMDIKNRKEYLSNDENWTDVAQMDDAKAIFNSKLSNVLSRYWRFCVDGGASSYYPQYTELQILGQRLSNDVANTLKD

SEQ ID NO: 5 - protein, 834 aa, synthetic construct
EEKTVQTGKTDQQVGAKLVQEIREGKRGPLYAGYFRTWHDRASTGIDGKQQHPENTMAEVPKEVDILFVFHDHTASDSPFWSELKDSYVHKLHQQGTALVQTIGVNELNGRTGLSKDYPDTPEGNKALAAAIVKAFVTDRGVDGLDIDIEHEFTNKRTPEEDARALNVFKEIAQLIGKNGSDKSKLLIMDTTLSVENNPIFKGIAEDLDYLLRQYYGSQGGEAEVDTINSDWNQYQNYIDASQFMIGFSFFEESASKGNLWFDVNEYDPNNPEKGKDIEGTRAKKYAEWQPSTGGLKAGIFSYAIDRDGVAHVPSTYKNRTSTNLQRHEVDNISHTDYTVSRKLKTLMTEDKRYDVIDEKDFPDKALREAVMAQVGTRKGDLERFNGTLRLDNPAIQSLEGLNKFKKLAQLDLIGLSRITKLDRSVLPANMKPGKDTLETVLETYKKDNKEEPATIPPVSLKVSGLTGLKELDLSGFDRETLAGLDAATLTSLEKVDISGNKLDLAPGTENRQIFDTMLSTISNHVGSNEQTVKFDKQKPTGHYPDTYGKTSLRLPVANEKVDLQSQLLFGTVTNQGTLINSEADYKAYQNHKIAGRSFVDSNYHYNNFKVSYENYTVKVTDSTLGTTTDKTLATDKEETYKVDFFSPADKTKAVHTAKVIVGDEKTMMENLAKGAKVIGTSGDFEQAKKIFDGEKSDRFFTWGQTNWIAFDLGEINLAKEWRLFNAETNTEIKTDSSLNVAKGRLQILKDTTIDLEKMDIKNRKEYLSNDENWTDVAQMDDAKAIFNSKLSNVLSRYWRFCVDGGASSYYPQYTELQILGQRLSNDVANTLKD

SEQ ID NO: 6 - protein, 834 aa, synthetic construct
EEKTVQTGKTDQQVGAKLVQEIREGKRGPLYAGYFRTWHDRASTGIDGKQQHPENTMAEVPKEVDILFVFHDHTASDSPFWSELKDSYVHKLHQQGTALVQTIGVNELNGRTGLSKDYPDTPEGNKALAAAIVKAFVTDRGVDGLDIDIEHEFTNKRTPEEDARALNVFKEIAQLIGKNGSDKSKLLIMDTTLSVENNPIFKGIAEDLDYLLRQYYGSQGGEAEVDTINSDWNQYQNYIDASQFMIGFSFFEESASKGNLWFDVNEYDPNNPEKGKDIEGTRAKKYAEWQPSTGGLKAGIFSYAIDRDGVAHVPSTYKNRTSTNLQRHEVDNISHTDYTVSRKLKTLMTEDKRYDVIDEKDFPDKALREAVMAQVGTRKGDLERFNGTLRLDNPAIQSLEGLNKFKKLAQLDLIGLSRITKLDRSVLPANMKPGKDTLETVLETYKKDNKEEPATIPPVSLKVSGLTGLKELDLSGFDRETLAGLDAATLTSLEKVDISGNKLDLAPGTENRQIFDTMLSTISNHVGSNEQTVKFDKQKPTGHYPDTYGKTSLRLPVANEKVDLQSQLLFGTVTNQGTLINSEADYKAYQNHKIAGRSFVDSNYHYNNFKVSYENYTVKVTDSTLGTTTDKTLATDKEETYKVDFFSPADKTKAVHTAKVIVGDEKTMMVNLAEGATVIGGSADPVNARKVFDGQLGSETDNISLGWDSKQSIIFKLKEDGLIKHWRFFNDSARNPETTNKPIQEASLQIFNIKDYNLDNLLENPNKFDDEKYWITVDTYSAQGERATAFSNTLNNITSKYWRVVFDTKGDRYSSPVVPELQILGYPLPNADTI

SEQ ID NO: 7 - DNA, 2682 bp, synthetic construct
  source 1..2682: mol_type = other DNA
gaagaaaaaaccgtgcaagtgcagaaaggcctgccgagcattgatagcctgcattatctgagcgaaaacagcaaaaaggaatttaaagaagaactgagcaaagcgggccaagaaagtcagaaagtgaaagaaattctggcgaaagcgcagcaagcggataaacaagcgcaagaactggcgaaaatgaaaattccggaaaaaattccgatgaaaccgctgcatggcccgctgtatggcggctattttcgcacctggcatgataaaacgagcgatccgaccgaaaaagataaagtgaacagcatgggcgaactgccgaaagaagtggatctggcgtttatttttcatgattggaccaaagattatagcctgttttggaaagaactggcgaccaaacatgtgccgaaactgaacaaacaaggcacccgcgtgattcgcaccattccgtggcgctttctggcgggcggcgataacagcggcattgcggaagatacgagcaaatatccgaacaccccggaaggcaacaaagcgttagcgaaagcgattgtggatgaatatgtgtataaatataacctggatggcctggatgtggatgtggaacatgatagcattccgaaagtggataaaaaagaagataccgcgggcgtggaacgcagcattcaagtgtttgaagaaattggcaaactgattggcccgaaaggcgtggataaaagccgcctgtttattatggatagcacctatatggcggataaaaacccgctgattgaacgcggcgcgccgtatattaacctgttactggtgcaagtgtatggcagccaaggcgaaaaaggcggctgggaaccggtgagcaaccgcccggaaaaaacgatggaagagcgctggcaaggctatagcaaatatattcgcccggaacagtatatgattggctttagcttttatgaagaaaacgcgcaagaaggcaacctgtggtatgatattaacagccgcaaagatgaagataaagcgaacggcattaacaccgatattaccggcacccgcgcggaacgctatgcgcgctggcagccgaaaaccggcggcgtgaaaggcggcatttttagctatgcgattgatcgcgatggcgtggcgcatcagccgaaaaaatatgcgaaacagaaagaatttaaagatgcgaccgataacatttttcatagcgattatagcgtgagcaaagcgctgaaaaccgtgatgctgaaagataaaagctatgatctgattgatgaaaaagattttccggataaagcgctgcgcgaagcggtgatggcgcaagtgggcacccgcaaaggcgatctggaacgctttaacggcaccctgcgcctggataacccggcgattcagagcctggaaggcctgaacaaatttaaaaaactggcgcagctggatctgattggcctgagccgcattaccaaactggatcgcagcgtgctgccggcgaacatgaaaccgggcaaagataccctggaaaccgtgctggaaacctataaaaaagataacaaagaagaaccggcgaccattccgccggtgagcctgaaagtgagcggcctgaccggcctgaaagaactggatctgagcggctttgatcgcgaaaccctggcgggcctggatgcggcgaccctgacgagcctggagaaagttgatattagcggcaacaaactggatctggcgccgggcaccgaaaaccgtcagatttttgataccatgctgagcaccattagcaaccatgtgggcagcaacgaacagaccgtgaaatttgataaacagaaaccgaccggccattatccggatacctatggcaaaacgagcctgcgcctgccggtggcgaacgagaaagtggatctgcaaagtcagctgctgtttggcaccgtgaccaaccaaggcaccctgattaacagcgaagcggattataaagcgtatcagaaccataaaattgcgggccgcagctttgtggatagcaactatcattataacaactttaaagtgagctatgaaaactataccgtgaaagtgaccgatagcaccctgggcaccacgaccgataaaaccctggcgaccgataaagaagagacctataaagtggatttttttagcccggcggataaaaccaaagcggtgcataccgcgaaagtgattgtgggcgatgaaaaaaccatgatggagaacctggccaaaggcgcgaaggtgattggcacgagcggcgattttgaacaagcgaaaaaaatttttgatggcgaaaaaagcgatcgcttttttacctggggtcagaccaactggattgcgtttgatctgggcgaaattaacctggcgaaagaatggcgcctgtttaacgcggaaaccaacaccgaaattaaaaccgatagcagcctgaacgtggcgaaaggccgcctgcagatcctgaaagataccaccattgatctggaaaaaatggatattaaaaaccgcaaagaatatctgagcaacgatgaaaactggaccgatgtggcgcagatggatgatgcgaaagcgatctttaacagcaaactgagcaacgtgctgagccgctattggcgcttttgcgtggatggcggcgcgagcagctattatccgcagtataccgaactgcagattctgggtcagcgcttaagtaacgacgtggccaacaccctgaaagat

SEQ ID NO: 8 - DNA, 2430 bp, synthetic construct
  source 1..2430: mol_type = other DNA
gaagaaaaaaccgtgcagaccggcaaaaccgatcaacaagtgggcgcgaaactggtgcaagaaattcgcgaaggcaaacgcggcccgctgtatgcgggctattttcgcacctggcatgatcgcgcgagcaccggcattgatggcaaacagcagcatccggaaaacaccatggcggaagtgccgaaagaagtggatattctgtttgtgtttcatgatcataccgcgagcgatagcccgttttggagcgaactgaaagatagctatgtgcataaactgcatcagcaaggcaccgcgctggtgcagaccattggcgtgaacgaactgaacggccgcaccggcctgagcaaagattatccggataccccggaaggcaacaaagcgctggcggccgcgattgtgaaagcgtttgtgaccgatcgcggcgtggatggcctggatattgatattgaacatgaatttaccaacaaacgcaccccggaagaagatgcgcgcgcgctgaacgtgtttaaagaaattgcgcagctgattggcaaaaacggcagcgataaaagcaaattactgattatggataccaccctgagcgtggaaaacaacccgatttttaaaggcattgcggaagatctggattatctgctgcgtcagtattatggcagccaaggcggcgaagcggaagtggataccattaacagcgattggaatcagtatcagaactatattgatgcgagtcagtttatgattggctttagcttttttgaagaaagcgcgagcaaaggcaacctgtggtttgatgtgaacgaatatgatccgaacaacccggaaaaaggcaaagatattgaaggcacccgcgcgaaaaaatatgcggaatggcagccgagcaccggcggcctgaaagcgggcatttttagctatgcgattgatcgcgatggcgtggcgcatgtgccgagcacctataaaaaccgcacgagcaccaacctgcagcgccatgaagtggataacattagccataccgattataccgtgagccgcaaactgaaaaccctgatgaccgaagataaacgctatgatgtgattgatcagaaagatattccggatccggcgctgcgcgaacagattattcagcaagtgggtcagtataaaggcgatctggaacgctataacaaaaccctggtgctgaccggcgataaaattcagaacctgaaaggcctggagaaactgagcaaactgcagaaactggaactgcgtcagctgagtaacgtgaaagagattaccccggaactgctgccggaaagcatgaaaaaagatgcggaactggtgatggtgggcatgaccggcctggaaaaattaaatttaagcggcctgaaccgtcagaccctggatggcattgatgtgaacagcattacccatctgacgagctttgatattagccacaacagcctggatctgagcgaaaaaagcgaagatcgcaaactgctgatgaccctgatggaacaagtgagcaaccatcagaaaattaccgtgaaaaacaccgcgtttgacaaacagaaaccgaccggccattatccggacacgtacggcaaaacgagcctgcgcctgccggtggcgaacgaaaaagtggatctgcagagtcagctgctgtttggcaccgtgaccaaccaaggcaccctgattaacagcgaagcggattataaagcgtatcagaaccataaaattgcgggccgcagctttgtggatagcaactatcattataacaactttaaagtgagctatgaaaactataccgtgaaagtgaccgatagcaccctgggcaccacgaccgataaaaccctggcgaccgataaagaagaaacctataaagtggatttttttagcccggcggataaaaccaaagcggtgcataccgcgaaggtgattgtgggcgatgaaaaaaccatgatggaaaacttagcgaagggcgcgaaagtgattggtacgagcggcgattttgaacaagcgaaaaaaatttttgatggcgaaaagagcgatcgcttttttacctggggtcagaccaactggattgcgtttgatctgggcgaaattaacctggcgaaagaatggcgcctgtttaacgcggaaaccaacaccgaaattaaaaccgatagcagcctgaacgtggcgaaaggccgcctgcagattttaaaagataccaccattgatctggaaaaaatggatattaaaaaccgcaaagaatatctgagcaacgatgaaaactggaccgatgtggcgcagatggatgatgcgaaagcgatttttaacagcaaactgagcaacgtgttaagccgctattggcgcttttgcgtggatggcggcgcgagcagctattatccgcagtataccgaactgcagattctgggtcagcgcctgagcaacgacgtggcgaacaccctgaaagat

SEQ ID NO: 9 - DNA, 2502 bp, synthetic construct
  source 1..2502: mol_type = other DNA
gaagaaaaaaccgtgcagaccggtaaaaccgatcagcaggttggcgctaaactggtgcaggaaattcgcgaaggtaaacgtggtccgctgtacgcgggttacttccgtacctggcacgatcgcgcgtcgaccggtatcgacggtaaacagcagcacccggaaaacaccatggcagaagtcccgaaagaagttgacatcctgttcgttttccatgatcacactgccagcgatagcccgttctggtctgaactgaaagacagctacgtgcacaaactgcaccagcagggtaccgcgctggtgcagaccattggcgttaacgaactgaacggccgtaccggcctgagcaaagattacccggacacgccggaaggcaacaaagcactggcagctgcgatcgtgaaagccttcgttacggaccgcggcgttgatggcctggatattgatatcgaacatgaattcactaacaaacgtaccccggaagaagatgcgcgtgcgctgaacgttttcaaagaaatcgcacagctgatcggcaaaaacggctctgataaatctaaactgctgatcatggataccaccctgtccgttgaaaataacccgatttttaaaggtatcgccgaggatctggattatcttctgcgtcagtattacggctcccagggtggcgaagccgaagttgataccattaacagcgattggaaccagtaccagaactacatcgatgcatctcagttcatgatcggcttctccttcttcgaagaatccgcgagcaaaggtaacctgtggtttgatgttaacgagtatgacccgaacaacccggaaaaaggtaaagacatcgaaggtacccgtgccaaaaaatacgcggaatggcagccgtctaccggcggcctgaaagcgggtatcttcagctacgctatcgaccgcgacggcgtcgctcacgtgccatctacctataaaaaccgtacctccaccaacctgcagcgtcacgaagtcgataacattagccacactgattacaccgtgagccgtaaactgaaaaccctgatgaccgaagataaacgttacgacgttattgacgaaaaagactttccggacaaggccctgcgcgaagcagttatggcccaggttggcacccgtaaaggcgacctggaacgcttcaatggtacactgcgcctggataatccggccattcagagtctggaaggcctgaataaatttaaaaagctggcccagctggatctgatcggtctgagccgcatcacaaagctggaccgtagcgtgctgcctgcaaacatgaagccgggcaaagacacactggaaaccgtgctggaaacctataaaaaagacaataaagaagagcctgcaaccattccgcctgttagcctgaaagtgagcggcctgaccggtctgaaggaactggacctgagcggtttcgaccgtgaaaccctggcaggtctggatgcagccacattaacaagtttagaaaaagttgacatcagcggcaataaactggacctggcaccgggcaccgagaaccgccagatcttcgacaccatgctgagcaccatcagcaatcatgttggcagcaatgaacagaccgtgaaatttgacaaacagaagccgaccggccactatccggacacctacggcaaaacaagcctgcgcctgcctgtggccaacgaaaaagtggatctgcagagccagctgctgttcggtaccgttaccaaccagggtaccctgatcaatagtgaagcagactataaagcataccagaatcataagatcgccggccgtagctttgtggatagcaactatcactacaacaatttcaaggtgagctatgaaaactacacggttaaagtgaccgatagcacactgggtaccacaaccgataaaacactggccaccgataaagaggagacatacaaagtggacttctttagcccggccgacaaaaccaaagcagtgcacaccgccaaagttattgtgggtgacgaaaaaaccatgatggaaaacctggctaaaggcgctaaagttattggtacttctggcgacttcgaacaggctaagaaaatcttcgacggcgaaaaaagcgatcgcttcttcacctggggccagaccaactggatcgcgtttgatctgggtgaaattaacctggcgaaagagtggcgtttgttcaacgcggaaaccaacactgaaatcaaaaccgacagcagcctgaacgttgcgaaaggtcgtctgcagatcctgaaagacaccaccatcgacctggaaaaaatggacatcaaaaatcgtaaagaatatctgagcaacgatgaaaactggaccgacgtggcacagatggatgatgctaaagctatcttcaactctaaactgtccaacgttctgagccgttattggcgcttctgtgttgacggcggcgctagctcttactacccgcagtacaccgaactgcagatcctgggtcagcgcctgagcaacgatgttgcgaacaccctgaaagat

SEQ ID NO: 10 - DNA, 2502 bp, synthetic construct
  source 1..2502: mol_type = other DNA
gaagaaaaaaccgtgcagaccggcaaaaccgatcagcaagtgggcgcgaaactggtgcaagaaattcgcgaaggcaaacgcggcccgctgtatgcgggctattttcgcacctggcatgatcgcgcgagcaccggcattgatggcaaacagcagcatccggaaaacaccatggcggaagtgccgaaagaagtggatattctgtttgtgtttcatgatcataccgcgagcgatagcccgttttggagcgaactgaaagatagctatgtgcataaactgcatcagcaaggcaccgcgctggtgcagaccattggcgtgaacgaactgaacggccgcaccggcctgagcaaagattatccggacaccccggaaggcaacaaagcgctggcggccgcgattgtgaaagcgtttgtgaccgatcgcggcgtggatggcctggatattgatattgaacatgaatttaccaacaaacgcaccccggaagaagatgcgcgcgcgctgaacgtgtttaaagaaattgcgcagctgattggcaaaaacggcagcgataaaagcaaactgctgattatggataccaccctgagcgtggaaaacaacccgatttttaaaggcattgcggaagatctggattatctgctgcgtcagtattatggcagccaaggcggcgaagcggaagtggataccattaacagcgattggaatcagtatcagaactatattgatgcgagtcagtttatgattggctttagcttttttgaagaaagcgcgagcaaaggcaacctgtggtttgatgtgaacgaatatgatccgaacaacccggaaaaaggcaaagatattgaaggcacccgcgcgaaaaaatatgcggaatggcagccgagcaccggcggcctgaaagcgggcatttttagctatgcgattgatcgcgatggcgtggcgcatgtgccgagcacctataaaaaccgcacgagcaccaacctgcagcgccatgaagtggataacattagccataccgattataccgtgagccgcaaactgaaaaccctgatgaccgaagataaacgctatgatgtgattgatgaaaaagattttccggataaagcgctgcgcgaagcggtgatggcgcaagtgggcacccgcaaaggcgatctggaacgctttaacggcaccctgcgcctggataacccggcgattcagagcctggaaggcctgaacaaatttaaaaaactggcgcagctggatctgattggcctgagccgcattaccaaactggatcgcagcgtgctgccggcgaacatgaaaccgggcaaagataccctggaaaccgtgctggaaacctataagaaagataacaaagaagaaccggcgaccattccgccggtgagcctgaaagtgagcggcctgaccggcctgaaagaactggatctgagcggctttgatcgcgaaaccctggcgggcctggatgcggcgaccctgacgagcctggaaaaagtggatattagcggcaacaaactggatctggcgccgggcaccgaaaaccgtcagatttttgataccatgctgagcaccattagcaaccatgtgggcagcaacgaacagaccgtgaaatttgataaacagaaaccgaccggccattatccggatacgtatggcaaaacgagcctgcgcctgccggtggcgaacgaaaaagtggacctgcagagtcagctgctgtttggcaccgtgaccaaccaaggcaccctgattaacagcgaagcggattataaagcgtatcagaaccataaaattgcgggccgcagctttgtggatagcaactatcattataacaactttaaagtgagctatgaaaactataccgtgaaagtgaccgatagcaccctgggcaccacgaccgataaaaccctggcgaccgataaagaagaaacctacaaagtggatttttttagcccggcggataaaaccaaagcggtgcataccgcgaaagtgattgtgggcgatgaaaaaaccatgatggtgaacctggcggaaggcgcgaccgtgattggcggcagcgcggatccggtgaacgcgcgcaaagtgtttgatggtcagctgggcagcgaaaccgataatattagcctgggttgggatagcaaacagagcattatttttaaactgaaagaagatggcctgattaaacattggcgcttttttaacgatagcgcgcgcaacccggaaaccaccaacaaaccgattcaagaagcgagcctgcagatttttaacattaaagattataacctggataacctgctggaaaacccgaacaaatttgatgatgaaaaatattggattaccgtggatacctatagcgcgcaaggcgaacgcgcgaccgcgtttagcaacaccctgaacaacattacgagcaaatattggcgcgtggtgtttgataccaaaggcgatcgctatagcagcccggtggtgccggaactgcagattctgggctatccgctgccgaacgcggataccatt